European Patent Application EP 4 624 579 A1, published October 1, 2025. Title: MICROORGANISMS FOR PRODUCING PURINE NUCLEOTIDES AND PROCESS FOR PRODUCING PURINE NUCLEOTIDES USING THE SAME. Applicant: CJ CheilJedang Corporation. The sequence listing filed with the application follows.

SEQUENCE LISTING (58 sequences)

SEQ ID NO: 1 - DNA, 30 bp, synthetic construct
  source 1..30: mol_type = other DNA
gggtctagatcaccgcgcagctgacccacg

SEQ ID NO: 2 - DNA, 24 bp, synthetic construct
  source 1..24: mol_type = other DNA
atgaagtgtcaaactcctttggag

SEQ ID NO: 3 - DNA, 21 bp, synthetic construct
  source 1..21: mol_type = other DNA
atggatttcattgcccgccac

SEQ ID NO: 4 - DNA, 29 bp, synthetic construct
  source 1..29: mol_type = other DNA
gggtctagaaccgtggtagacggcgtaca

SEQ ID NO: 5 - DNA, 38 bp, synthetic construct
  source 1..38: mol_type = other DNA
aattcgagctcggtacccaggcacagccgacattacgg

SEQ ID NO: 6 - DNA, 35 bp, synthetic construct
  source 1..35: mol_type = other DNA
gtagcacatctgacgaatgtccaagtctaaggaaa

SEQ ID NO: 7 - DNA, 35 bp, synthetic construct
  source 1..35: mol_type = other DNA
ttagacttggacattcgtcagatgtgctacttgcc

SEQ ID NO: 8 - DNA, 35 bp, synthetic construct
  source 1..35: mol_type = other DNA
tgcgccattagcgtgttacttctcgcggctataga

SEQ ID NO: 9 - DNA, 35 bp, synthetic construct
  source 1..35: mol_type = other DNA
agccgcgagaagtaacacgctaatggcgcattgaa

SEQ ID NO: 10 - DNA, 35 bp, synthetic construct
  source 1..35: mol_type = other DNA
tgaattatccgcgtcttagatgccgttttctgccg

SEQ ID NO: 11 - DNA, 35 bp, synthetic construct
  source 1..35: mol_type = other DNA
gaaaacggcatctaagacgcggataattcagctgt

SEQ ID NO: 12 - DNA, 38 bp, synthetic construct
  source 1..38: mol_type = other DNA
cgactctagaggatccccgatgaagcgaacacttaaat

SEQ ID NO: 13 - DNA, 20 bp, synthetic construct
  source 1..20: mol_type = other DNA
ccagtacattgtcatgggat

SEQ ID NO: 14 - DNA, 20 bp, synthetic construct
  source 1..20: mol_type = other DNA
gattggcatatcgcaccgag

SEQ ID NO: 15 - DNA, 35 bp, synthetic construct
  source 1..35: mol_type = other DNA
gtacccggggatcctgaaatcatcagcgttggccc

SEQ ID NO: 16 - DNA, 38 bp, synthetic construct
  source 1..38: mol_type = other DNA
gaactcgtggtgatggtgactatatattcccttcgtcg

SEQ ID NO: 17 - DNA, 36 bp, synthetic construct
  source 1..36: mol_type = other DNA
ggaatatatagtcaccatcaccacgagttccttcag

SEQ ID NO: 18 - DNA, 35 bp, synthetic construct
  source 1..35: mol_type = other DNA
attctgggtagtcatgagtgtttcctttcgttggg

SEQ ID NO: 19 - DNA, 37 bp, synthetic construct
  source 1..37: mol_type = other DNA
cgaaaggaaacactcatgactacccagaattcttccg

SEQ ID NO: 20 - DNA, 35 bp, synthetic construct
  source 1..35: mol_type = other DNA
gcaggtcgactctagggaagactgcagagttgagc

SEQ ID NO: 21 - DNA, 38 bp, synthetic construct
  source 1..38: mol_type = other DNA
aattcgagctcggtaccccatttcgtgaccattagcgt

SEQ ID NO: 22 - DNA, 35 bp, synthetic construct
  source 1..35: mol_type = other DNA
attagcctgaaggaagatcatgccaatagcgccag

SEQ ID NO: 23 - DNA, 35 bp, synthetic construct
  source 1..35: mol_type = other DNA
gctattggcatgatcttccttcaggctaatctttt

SEQ ID NO: 24 - DNA, 35 bp, synthetic construct
  source 1..35: mol_type = other DNA
attctgggtagtcatcatatgtgtttcctttcgtt

SEQ ID NO: 25 - DNA, 35 bp, synthetic construct
  source 1..35: mol_type = other DNA
aaggaaacacatatgatgactacccagaattcttc

SEQ ID NO: 26 - DNA, 35 bp, synthetic construct
  source 1..35: mol_type = other DNA
ctttgtacttggtgaccaagagtcaggatgccgaa

SEQ ID NO: 27 - DNA, 35 bp, synthetic construct
  source 1..35: mol_type = other DNA
catcctgactcttggtcaccaagtacaaagagact

SEQ ID NO: 28 - DNA, 38 bp, synthetic construct
  source 1..38: mol_type = other DNA
cgactctagaggatccccggttaccgcgcattaggact

SEQ ID NO: 29 - DNA, 20 bp, synthetic construct
  source 1..20: mol_type = other DNA
taatcccccagctcaccggc

SEQ ID NO: 30 - DNA, 20 bp, synthetic construct
  source 1..20: mol_type = other DNA
tttggatgccgaggtcgtag

SEQ ID NO: 31 - DNA, 38 bp, synthetic construct
  source 1..38: mol_type = other DNA
tcgagctcggtacccgttgccgtatcagacatgctcag

SEQ ID NO: 32 - DNA, 38 bp, synthetic construct
  source 1..38: mol_type = other DNA
gattagcctgaaggaattgatttatctcgaccaaacag

SEQ ID NO: 33 - DNA, 38 bp, synthetic construct
  source 1..38: mol_type = other DNA
ggtcgagataaatcaattccttcaggctaatcttttcc

SEQ ID NO: 34 - DNA, 38 bp, synthetic construct
  source 1..38: mol_type = other DNA
cgatataagactccatcatatgtgtttcctttcgttgg

SEQ ID NO: 35 - DNA, 38 bp, synthetic construct
  source 1..38: mol_type = other DNA
aaaggaaacacatatgatggagtcttatatcggtagcc

SEQ ID NO: 36 - DNA, 38 bp, synthetic construct
  source 1..38: mol_type = other DNA
ctcataggtgccgaacttactcggagatttcgacctca

SEQ ID NO: 37 - DNA, 38 bp, synthetic construct
  source 1..38: mol_type = other DNA
cgaaatctccgagtaagttcggcacctatgagaatatg

SEQ ID NO: 38 - DNA, 39 bp, synthetic construct
  source 1..39: mol_type = other DNA
ctctagaggatccccggcaagtgtttcttggcgccattc

SEQ ID NO: 39 - DNA, 19 bp, synthetic construct
  source 1..19: mol_type = other DNA
gcgagggggaagaaaagta

SEQ ID NO: 40 - DNA, 18 bp, synthetic construct
  source 1..18: mol_type = other DNA
cgttgccctttttcttct

SEQ ID NO: 41 - protein, 952 aa, Corynebacterium stationis
MDFIARHLGPDATESKDMLARVGYDSVEALVTSAIPQSISITDALNMPQALSETDAQAKLRAYADKNVVLKSFYGQGYSDTITPAVIRRGLVEDAGWYTAYTPYQPEISQGRLESLLNFQTMVQDLTGLPIANASLLDEASAVAEAVGLMSRAVKKGRRVLLDARLHPQVLTVAAERARAIDLEVEIADLSNGVVGEDLVGAVVAYTGTEGDIFDPRAVIEEIHGRGGLVSVAADLLSLLLLEGPGSFGADIVIGSSQRFGVPLFFGGPHAAFMAVTDKLKRQMPGRLVGVSVDSEGRPAYRLALQTREQHIRRERATSNICTAQALLANVAAMYAVYHGPEGLKEIANHVHSLAASFAGAVTTQGLKITSSEFFDTVTVAGVDAASIKFSLEKAGYLVRTIGEDKVSVSFGESATQGDVTVLADAFGAAAVDNADFPLPEALTRTTEVLTHEIFNSIHSETQMMRYLRKLGDKDLALDRTMIPLGSCTMKLNPTAAMEPITWPEFANVHPYSPEYATQGWRELIEELEGWLAELTGYAKVSIQPNAGSQGELAGLLAIRRYHVANGDTNRDIVLIPASAHGTNAASATLANLRVVVVKTAEDGSIDLEDLDAKIAKHGQNMAGIMITYPSTHGVFDPEVREVCDKIHAAGGQVYIDGANMNALTGWAQPGKFGGDVSHLNLHKTFTIPHGGGGPGVGPIGVAEHLIPFLPTDAAADELDPANPTPVEQGVPITASQFGSAGVLPITWAYIAMTGGEGLTSATAHAILGANYLARELSDSFPILFTGNEGLVAHECILDLRALTDASGVTAADVAKRLIDFGFHAPTLAFPVAGTLMVEPTESEDIAELDRFIEAMRTIRAEIQEIIDGKIAYEDSVIRHAPYTAPSVSSDDWEYSFSREKAAWPVPSLRLNKYFPPVRRLDEAYGDRNLVCSCPPPEAFDFDADTDSTEEA

SEQ ID NO: 42 - DNA, 2859 bp, Corynebacterium stationis
  source 1..2859: mol_type = genomic DNA
atggatttcattgcccgccaccttgggccagatgccacagaatctaaggacatgctggcgcgtgtgggttatgacagcgtagaagcgcttgtcacctcagcaatcccccagtccattagcatcacggatgcgcttaatatgccgcaggcattgagtgagaccgacgcacaagccaagcttcgcgcttacgctgataaaaatgtcgtgctgaagtctttctacggccagggctactcagacaccatcacccctgctgttattcgccgcggtttggtagaagacgctggttggtacaccgcttataccccataccagccagaaatttcccagggtcgccttgagtcgctgctgaacttccagaccatggttcaagacctcaccggcttgcctattgcgaatgcttctttgctggatgaggcatcggcagttgctgaggccgtgggtttgatgtctcgtgcggtcaagaagggccgccgcgtactgctcgacgcccgtttgcacccacaggttctcaccgtggcggcggagcgtgcccgagcaattgacctcgaagttgagattgctgacttgagcaacggcgtggttggcgaagacctcgtcggcgcagtagttgcctacaccggtacggagggcgatatttttgacccacgtgctgttatcgaagaaatccatggccgcggcggacttgtttccgtcgcggctgacttgttgtccttgctgcttctggaaggcccaggctcgttcggtgcagacattgtcattggttcctcccaacgctttggtgtgccgctcttctttggtggcccacacgctgctttcatggcagtaactgacaagctaaagcgtcagatgccaggccgtttggtcggcgtatcggtcgattctgagggccgtcctgcttaccgcttggcgctgcagactcgtgaacagcacatccgccgtgaacgcgcgacgtcaaatatttgtaccgcgcaggcacttctggccaacgtggctgccatgtacgccgtctaccacggtccagaaggcttgaaggagattgctaaccacgtgcactccttggctgcttcctttgccggtgcagttactactcagggtctgaagattacttcctcggagttcttcgacaccgttaccgttgccggcgttgatgccgcatccattaagttcagcttggaaaaggccggatacctggtgcgcaccattggcgaggataaggtttctgtctccttcggtgagtccgcaacccaaggcgatgttactgtcttggcggacgcctttggtgccgctgcagtagataatgcagatttcccactgcctgaagcactcacccgcaccaccgaggtgctcacccacgaaatctttaactccattcactccgaaacccagatgatgcgttacctgcgcaagctcggtgataaggatctggctctagatcgcaccatgattcctttgggctcatgcaccatgaagctcaacccaaccgcagccatggaaccgatcacctggccagaattcgccaatgttcacccttactcccctgaatacgcaacccagggctggcgtgagctcattgaagagttggaaggctggttggctgagctgaccggctacgccaaggtttctatccaaccaaacgctggttcccagggcgagctagctggtcttttggctatccgccgctaccacgtcgcaaatggtgacaccaaccgcgatatcgtgttgattcctgcgtccgcgcacggcaccaacgctgcctccgcgaccctggcaaatctgcgcgttgttgtggttaagaccgccgaagacggctccatcgatctggaagatctcgatgcgaagatcgccaagcatggtcagaacatggccggaatcatgatcacctacccatccactcacggcgtctttgacccagaggttcgtgaagtctgcgacaagatccatgccgctggcggccaggtctacattgatggcgcaaacatgaatgctttgactggttgggctcagccgggcaagttcggtggcgatgtctcgcacttgaacctgcacaagactttcaccattccgcacggcggtggcggcccaggtgttggaccaattggtgtcgctgagcacctcattccattcctgccaacggatgctgcagctgatgagctggatcctgctaacccaaccccagtagaacagggcgttccaattactgcttcgcagtttggttccgctggtgttctgccgattacctgggcatacatcgcaatgaccggtggcgagggtctaacctccgctactgcacacgccatcttgggtgctaactaccttgcgcgcgaactctccgattccttcccaattctgttcaccggtaatgaaggtcttgttgcgcacgagtgcattttggatctgcgcgcgctaaccgatgcctcaggcgttactgcagcagacgttgccaagcgtttgatcgactttggcttccacgctcctaccctcgcattcccagtggctggcaccttgatggtggaacctactgagtctgaggatattgctgaactggatcgtttcattgaagcaatgcgcaccatccgtgcggagattcaggaaatcatcgatggcaagatcgcatatgaagattcggtcatccgccacgcaccttacaccgcaccgtcagtctcaagcgatgattgggagtactcctttagccgtgaaaaggccgcatggccagttccttcactgcgtttgaacaagtacttcccaccggtacgccgcctggatgaagcttacggcgaccgcaacctggtgtgctcctgcccaccgccagaggcattcgacttcgatgccgacaccgattccaccgaggaggcttaa

SEQ ID NO: 43 - protein, 367 aa, Corynebacterium stationis
MSELRQSPLHAEHEKLGASFTAFGPWNMPLKYGKELDEHHAVRNAVGMFDLSHMGEIWVNGPDAAAFLSYALISNMETVKNGKAKYSMIVAEDGGIIDDLISYRFSDTKFLVVPNAGNTDVVWEAFNQRIEGFDVELNNESLDVAMIALQGPNAAKVLVEQVAEESKEEVENLPYYAATMAKVADVDTIVARTGYTGEDGFELMIYNADATKLWQLFIDQDGVTPCGLASRDSLRLEAGMPLYGNELSRDITPVEAGMGVAFKKKTADFVGAEVLRQRLEEGPKQVIKALTSSERRAARTGAEIYAGEQLVGTVTSGQPSPTLGHPIALALVDTAANLEEGAEVEVDIRGKRYPFTVTKTPFYSREK

SEQ ID NO: 44 - DNA, 1104 bp, Corynebacterium stationis
  source 1..1104: mol_type = genomic DNA
atgtcagaactacgccagtccccactgcacgcagagcacgaaaagctcggcgcatcctttaccgcttttggcccttggaatatgccactaaagtacggcaaggagctcgatgagcaccacgcagtgcgtaatgcagtcggcatgtttgacctctcgcacatgggtgagatttgggtcaacggcccagacgccgctgcatttttgtcctatgcgctgatctccaacatggagaccgtgaaaaatggcaaggcgaagtactccatgattgttgctgaagacggcggcatcatcgatgacctaatttcctaccgtttctccgataccaagttcttggtagtgccaaacgctggcaacactgatgtggtttgggaagcttttaatcagcgcattgaaggcttcgatgtagaactcaacaatgagtccttggatgttgcgatgattgccctgcagggccccaatgctgccaaggttctagttgaacaggttgctgaagagtccaaggaagaagtagaaaaccttccttactatgccgcaaccatggccaaagtcgcagacgttgacaccatcgtcgcgcgcaccggctacaccggcgaagacggcttcgagctgatgatctacaacgccgatgcgaccaagctctggcagcttttcatcgaccaagatggtgttactccatgcggtttagcttcacgcgattccttgcgcttggaagctggcatgcctttgtacggcaatgagctttcccgcgatatcacccctgtcgaggcaggcatgggtgtggcgtttaagaagaagaccgctgacttcgtcggcgccgaggtcctgcgtcaacgcttggaagaaggccctaagcaagttatcaaggctttgacctcctctgagcgccgtgcagcgcgcaccggtgctgaaatctatgccggcgagcagttggtaggcaccgtaacttcgggtcagccatcgccgacgctgggacaccctattgccctggcactggtagatactgcagcaaacctcgaagaaggcgcagaagtagaagtggatattcgcggcaagcgttaccccttcaccgttaccaagacgcctttctatagccgcgagaagtaa

SEQ ID NO: 45 - protein, 129 aa, Corynebacterium stationis
MANLPAEFTYSEDHEWINAAQDAIVGKTVRIGITSVAADRLGEVVFAELPAVGDSVTAGETCGEVESTKSVSDLYSPVTGTVTAVNETVHDDYEIINNDPFGEGWLFEVEVEELGEVMTADEYAAENGI

SEQ ID NO: 46 - DNA, 390 bp, Corynebacterium stationis
  source 1..390: mol_type = genomic DNA
atggctaacctacctgcagaatttacttactccgaagaccacgagtggattaacgccgctcaggacgcaatcgttggcaaaactgttcgcatcggcatcacttctgttgccgcagaccgtcttggtgaggttgtcttcgctgagcttccagcagttggcgatagcgtcactgcaggtgaaacctgtggtgaggttgaatccaccaagtccgtttctgacctgtacagccctgtcaccggtaccgtgaccgctgtgaacgagacagtgcacgatgattatgaaatcatcaacaatgatcctttcggtgaaggttggctgtttgaggtcgaggttgaagaactcggcgaggttatgaccgctgatgaatacgcggcagaaaacggcatctaa

SEQ ID NO: 47 - protein, 433 aa, Corynebacterium stationis
MTTQNSSDAQYQEMRDLDPEVYAAINGEIARQRDTLEMIASENFVPRAVLQAQGSVLTNKYAEGYPGRRYYGGCEHVDIVEDLARDRAKALFGAEFANVQPHSGAQANAAVLASLINPGDKILGLSLAHGGHLTHGMKLNFSGKLYEVAAYEVDAETNRIDMDKLREQAIAEKPQVIIAGWSAYPRTLDFEAYRSIADEVGAYLWTDMAHFAGLVAADLYPNPVPHSDIVSTTVHKTLGGPRSGMILAKQDYAKKLNSAVFPGQQGGPLMHVVAAKAIAMKVAASEEFRDRQVRTLEGAKILAERLTTPEAKAAGVDVLTGGTDVHLVLADLRNSEMDGQQAEDLLHEVGITVNRNAVPNDPRPPMVTSGLRIGTSALATRGLDAEAFTEVADIIGTALTDGKNADTQKLRARVDKLAEQFPLYEGLEDWKIV

SEQ ID NO: 48 - DNA, 1302 bp, Corynebacterium stationis
  source 1..1302: mol_type = genomic DNA
atgactacccagaattcttccgatgctcagtaccaggaaatgcgtgacttagacccagaggtctatgcagcaattaacggtgaaattgctcgtcagcgcgataccctggagatgattgcgtcggagaactttgttcctcgtgcagtcttgcaggcacagggttccgtccttaccaacaagtacgcagagggctacccaggtcgccgctactacggtggatgtgagcacgtcgatatcgtcgaagatctggcgcgtgaccgcgctaaggctctgttcggcgctgagtttgccaatgtacagccacactccggtgcacaggcaaacgctgccgtccttgcttctcttatcaacccaggcgataagatcttgggcctttctttggctcacggtggtcacctgacccacggcatgaagctgaacttctccggcaagctctacgaagtagctgcctacgaagtcgatgcagaaaccaaccgtatcgacatggacaagctgcgtgagcaggctattgcagaaaagccacaggtcatcatcgctggctggtctgcatacccacgcactctggattttgaagcataccgttccatcgcggatgaagtgggggcttacctgtggaccgatatggcacactttgctggtctcgttgccgctgatctgtacccaaatccagttccacactctgacattgtttccaccaccgtgcacaagaccctgggcggtcctcgctccggcatgatcctggctaagcaggactacgctaagaagctcaactctgcagtcttcccaggccagcagggtggccctttgatgcatgtggttgcagcgaaggcaattgccatgaaggttgctgcttccgaagaattccgtgaccgtcaggtccgtactctggaaggcgcgaagattcttgctgagcgcttgaccactcctgaggcaaaggcagcaggcgttgacgttctcactggcggcaccgacgtgcacttggttcttgcggacctgcgcaattctgagatggatggccagcaggcagaagacctcctgcacgaggtcggcatcaccgttaaccgcaacgcggttccaaacgatccacgtccaccaatggtgacctctggtctgcgtatcggtacttccgctctggctacccgcggcctggatgcagaagcattcaccgaggtggcagacatcatcggcaccgcgcttaccgatggcaagaacgccgatacccagaagctgcgcgcacgcgtggacaagcttgctgagcagttcccactctacgagggcttggaagactggaagatcgtctaa

SEQ ID NO: 49 - protein, 422 aa, Corynebacterium stationis
LESYIGSPLTSNAVRVLMLGGGELAKGLVGAFQNLGLEVHVVDRYEGSPAQQVAHFSYTADIDDEKAVLDLVEHIKPAYVVPEIEGVADEALHALHDDSAVTVVPTARACELTSDRKKLREVAESLGLPTTAYKVVETFDALKEAVNELGLPCIIKPDVATSGRGHVLVKDEDQLKDAWDNVRRGKKNSWVVAERFVDFDYEVIIMAVRSIDPETGKLATWFSEPIGYEHARGNLVDCWQPKTMSQRAFENARSVAARISNELGGRGIFAVELFVAGDDIYFSSVTPRPSDKAMLTEATQRFSQYELHARAILGLPIDITLVSPGASSLLHATEEIDEVTYSGVEEALQVAETDVRLFGKPSAYPGRRMGLIMATADDVSEARDRAAIAASKITISAAPRLVPEPELTSEKELSPDEVEISE

SEQ ID NO: 50 - DNA, 1269 bp, Corynebacterium stationis
  source 1..1269: mol_type = genomic DNA
ttggagtcttatatcggtagccccctgacctcgaatgctgttcgggttctcatgctcggcggcggtgagctggccaaaggtttggtgggcgcgtttcagaatttgggcttggaagtccacgttgtcgaccgctatgaggggtctccagcacagcaggttgcacactttagctacaccgcagatatcgatgatgaaaaggccgtgctcgatttagttgagcacatcaagccggcttatgtcgtgccagaaatcgagggcgtagcagatgaggctttgcatgcgcttcacgatgactccgctgtcaccgttgtgcccaccgcccgggcgtgtgagcttaccagcgaccggaagaagctacgcgaagtcgcagaaagcctcggcttgccgacgaccgcgtacaaggtcgtagaaaccttcgacgctttgaaagaagcggtgaacgagctcggtttgccgtgcattattaagccggatgttgcaacctctggacgcgggcatgtgctggtcaaagacgaagaccaactcaaagacgcgtgggataatgtgcgtcgcggcaagaagaactcctgggttgtcgccgaacgctttgtggattttgactatgaagtcatcatcatggcggtgcgctcgattgacccggaaacgggcaagctggcaacgtggttctcagagccgattggttatgagcatgcgcgcggcaacctcgtggactgctggcagccaaagacgatgagccagcgtgcttttgaaaatgcacgttcggttgcagcgcgtatttctaacgaactcggcggccgcggcatcttcgcggtggagctgtttgtcgcgggcgacgatatctacttctcctcggtgaccccgcgtccttctgataaagcgatgctgaccgaagccacccaacgcttttcgcagtatgaattgcacgcgcgcgccattttgggcctgccgatcgacatcacgcttgtctcaccgggcgctagctctttgttgcacgcgaccgaagagatcgacgaagttacctactcgggcgttgaagaagccctgcaggttgcagaaaccgatgtgcgcctattcggcaagccttcggcataccctggccgacgcatggggttgatcatggccaccgccgacgatgtctccgaagcacgcgaccgcgctgcgatcgcggcatcgaagatcacgattagcgccgccccaaggttagttcctgaaccagaactaacctctgaaaaagagttatcccccgatgaggtcgaaatctccgagtaa

SEQ ID NO: 51 - protein, 470 aa, Corynebacterium stationis
VTISVIDIFSVGVGPSSSHTVGPMRAAKTFMESLPHAPAKVHTELRGSLSATGKGHATDRAVILGLAGWAPLTVPIDAKPLAGSFIPSEGTVEGPAGSVQYSIAFNNKPVPEHPNCLIFSAWDENGEEIATNMEYFSVGGGFVLSRAELDAQLQATHEVPAGMAAAQNNDNAIPYDFSTGDQLLELCDEHDMTIWEIVAANEAVIHREDGGLAKVNAHLDLVWDVMRECVTDGIATKGILPGGLQVNRRAPQLYSQLLEHQDDTASGFSAMEWVNLYALAVNEQNAAGGRVVTAPTNGACGIIPAVLHYARDFLPDFTRETARRFLLTAGAIGMIIKQNASISGAEVGCQGEVGSASSMAAAGLAEILGSSPAQIENAAEIALEHNLGLTCDPVGGLVQIPCIERNAIGAVKSINSARLARMGEGTHYVTLDNAVQTMAETGRDMLTKYKETSIGGLAKTLGLSVSQVEC

SEQ ID NO: 52 - DNA, 1413 bp, Corynebacterium stationis
  source 1..1413: mol_type = genomic DNA
gtgaccattagcgtcattgacatcttttcagtaggcgtggggccttcgtcctcccacaccgttggccccatgcgtgcagcgaaaacctttatggaatctttgccgcatgctcctgccaaagtacatactgagctgcgtggttcactctcagccacgggtaaaggccacgccaccgaccgcgccgtcattttaggccttgccggatgggcgccacttaccgtacctattgacgctaagccgcttgccggcagttttatcccttctgaaggcacagtcgaaggccccgccggcagcgtgcagtattccattgcgttcaacaacaagccggtgcctgagcacccgaactgtttgatatttagcgcctgggatgaaaatggtgaagaaatcgctaccaatatggagtacttctccgtgggcggcggctttgttctctcacgtgcagagctcgatgcgcagctgcaagccacccacgaagttccggcgggtatggcggctgcgcaaaataatgacaacgcaatcccctatgacttcagcaccggtgatcagctcctagagttgtgcgatgagcacgacatgacaatctgggaaatcgtcgctgccaatgaagcagttattcaccgtgaagatggtgggctggccaaggtcaacgcgcacttggatctggtgtgggatgtcatgcgtgagtgtgttactgatggcattgctaccaaggggattttgcccggtggtctgcaggttaatcgtcgtgctccgcaactttatagtcaattgcttgaacaccaagatgatactgcgtcaggcttttctgccatggagtgggtcaacctctatgcactagccgtcaacgagcaaaatgctgccggtggccgcgtggtcactgctccaactaacggtgcctgcggaatcattcccgcggtcttgcactatgcacgagacttcctccccgatttcactcgtgagacagcccggcgttttctgctcaccgctggcgctattggcatgatcatcaagcagaatgcttctatctctggcgctgaggttggctgccaaggagaagtcggctcggcatcgtcaatggctgctgccgggttggctgagattttaggctcgagtccagcacagatcgaaaatgcggcagaaatagcactcgagcacaatctcggtctaacctgcgatccggtcggcggcttggtgcagattccgtgcatcgagcgcaatgcgattggcgcagtaaagtctattaactccgcacgccttgcccgcatgggtgaaggcacgcattacgtcaccctcgataatgctgtgcagacaatggccgagaccggccgagacatgctcaccaagtacaaagagacttcgatcggtggcttggctaagaccctgggactatctgtctcccaggtggagtgctaa

SEQ ID NO: 53 - protein, 361 aa, Corynebacterium stationis
MTATTNHLTENSHAHGYDHYQRMAFFTDTSVCIGCKACEVACKEWNRNPVEGYNLTGNSYDNTGALGANTWRHVAFIEQDNERITKAREEGAKLVSLGMPTIGTSPVDAAPNPASADTTPPDTDTFRWLMSSDVCKHCTNAGCLDVCPTGALFRTEFGTVVVQDDVCNGCGTCVAGCPFGVIERREDGGVSLKANHVEAQEVPEHAGINVFKKLKQLRPQGPDHVPGETMPIKNIGVAQKCTMCYDRLKVGEQPACSKTCPTESIQFGTYENMLAAAQARVAELHRQGQTEARLYGANNEDGVGGTGSIFLLLDSPEVYGLPPDPRVPTADLPAMAKTFAKAVGAMGVAVAASFLVDRGGT

SEQ ID NO: 54 - DNA, 1086 bp, Corynebacterium stationis
  source 1..1086: mol_type = genomic DNA
atgacggctacgaccaatcacctaacagaaaattcgcacgcgcacggctacgaccattaccagcgcatggcctttttcaccgatacttcggtgtgcattggctgtaaggcttgcgaggtggcctgtaaggagtggaaccgcaacccggttgagggctataacctgacgggtaattcctacgacaacaccggcgcgctgggcgcgaatacctggcgacacgtagcatttattgagcaagacaacgagcgcatcaccaaagcgcgtgaagaaggtgccaagctggtctcgctgggcatgccgacgattggcacttcgcctgtcgatgcagccccgaatcctgcctccgccgataccacgccgccggatactgatactttccgttggctgatgtcttctgatgtctgcaagcactgcaccaacgctggctgcctggatgtgtgcccaaccggtgctttatttcgcaccgaatttggcaccgtcgtggtccaagatgatgtctgcaatggctgcggcacctgcgttgccgggtgcccgttcggtgttattgagcgccgtgaagacggcggtgtttcgctaaaagccaaccacgtcgaagcccaagaagtccctgaacacgcgggcattaacgtgtttaagaagctcaaacagctgcgcccgcaaggaccggatcacgtcccgggtgagaccatgccgattaaaaatattggcgtggctcaaaagtgcaccatgtgctacgaccgcctgaaagtcggcgagcagccagcgtgttccaagacatgcccgacggagtccatccagttcggcacctatgagaatatgctggccgctgcgcaagcgcgcgtggctgagctacaccgtcaaggccagactgaggcacgactgtacggcgcaaataacgaagacggcgtcggcggaacgggctccatcttcttgctgctggattccccggaagtctacggtcttccaccagatccgcgtgtgccgactgcagatttgcccgcaatggcgaagactttcgccaaggccgttggcgccatgggcgttgccgtggcagcgtcctttttagttgatagaggagggacctag

SEQ ID NO: 55 - protein, 923 aa, Corynebacterium stationis
LGTSFGRGGATQPLQDMANADCILIQGSNMAECHPVGFQWVVEAKKRGARVIHVDPRYTRTSAFANRHVAIRGGTDVVLLGALIKYMIDNDLYFHDYVVNYTNASSIISPDFRDTEDLDGLFSGYNPETGKYITDSWQYVQKPEGAWWNIERDETLQDPNTVFQILKRHYSRYTPEIVEETCGISQEDFHYLAESIAQNSNPERTTVFAYALGFTQQTLGVQFIRAAAILQLLMGNVGRPGSGIMALRGHASIQGSTDIPTLFNNLPGYLPMPHADHGDWKGFLDAIAKEDQKGFWGLRENYAVSLMKSYWGENATKDNDWGWNYMPRINGAHSTYETLMGMLDGIVEGYIVFGQNPAVAQSNGGMQRRGLASLKWLVVRDFQEIETASFWYDSPEIKTGELKTEDIGTEVFLLPAATHVEKAGTFTQTQRMLQWRFQATNPPGDAKSDLWFFYQMGKRIREKLAGSTDPMDAPLLAIDWNYEETEHGEPDPEDVLREINGYYLDGPKKGQLLPGFTEMKPDGTTSGGCWIYSGVFKDNINQSARKVSGASQNEVALEWGWVWPSNRRMLYNRASAAPDGTPWSERKKYIWWDAEAGRWTGDDVPDFPVNLDPSYRAPVDATGPAALDGTDAFIMQADGRGWLFVPKGLSDGPLPTHYEPHESPARNILYSQQQSPTRLTIKRPDNLSKPMAGEPGSEVYPVVFSTYRLTEMYTSGAMSRRLPYLAELQPDLFVEVDPVLAQKRGLENGGWATIISPRGVIEARVLVTERMESMTINGKDFHQIGLPFHYGQSSSSPVTGDGANDLLGLTLEPNVFIQNSKVGACEIKAGRRPRGKARLEMLKEYQRRAGLTLDTGNELIDPDAQQLEATSTIDLFIPNGVDKETVETSTSEPGAADGSAHHGSAMGEVPNSEPKDTEGGEKQ

SEQ ID NO: 56 - DNA, 2772 bp, Corynebacterium stationis
  source 1..2772: mol_type = genomic DNA
ttgggaacctcgtttggccgcggtggcgcaactcagccactgcaggatatggcaaatgccgactgcatcctgattcagggctcgaatatggccgagtgccatcctgtgggtttccagtgggtagtcgaagctaaaaagcgcggggcgcgcgtaattcacgtggatcctcgctatacccgtacctcggcgtttgcgaaccggcacgtagcgatccgtggcggcaccgatgtggtgcttcttggcgcacttatcaagtacatgatcgacaatgatctgtattttcacgactatgtggtcaattacacgaacgcgtcgtcgatcatttctcccgacttccgggacacggaagacctagacggcctcttttctggctacaacccagaaaccggtaagtacatcacggactcgtggcagtacgtgcaaaagcccgaaggtgcgtggtggaatatcgagcgtgatgagactttgcaggacccgaatacggtcttccagattctcaagcgccactattcccgctataccccggaaatcgtggaagagacctgcggtatctcccaggaggacttccattatctagcggagtcgattgcacagaactccaatccagagcgcactacagtctttgcctatgctttgggctttacgcagcaaaccttaggcgtgcagttcattcgtgccgcggccatcttgcaactgctgatgggcaacgtgggccgcccgggctcaggcatcatggcgctgcgtggacacgcttccattcagggctcgacagatatcccgacgctgtttaataacttgccgggttacttgccgatgcctcatgccgaccatggcgactggaaaggattcttggacgcgattgccaaggaagaccagaagggtttctggggtctgcgtgaaaactatgccgtgagcttgatgaagtcctattggggcgagaatgccaccaaggacaatgactggggctggaactacatgccgcgcatcaacggtgcgcactccacctatgaaaccttgatgggcatgctcgacggcatcgtcgaaggctatatcgtcttcggacaaaacccagcggtcgctcaatccaacggcggcatgcaacgccgcggattggcgtctttgaagtggttggttgttcgtgacttccaggaaattgagacagcgtcattctggtacgactcaccagagatcaagactggtgaactcaagaccgaagatattggcaccgaggtcttccttcttcctgcagcaacgcacgtagaaaaggccggtacctttacccaaacccagcgcatgctgcagtggcgtttccaggccacaaatccaccaggcgatgccaagagcgatctgtggttcttctaccagatgggcaagcgcattcgcgaaaagcttgctggttctactgatccgatggacgcgccattgttggccatcgactggaactacgaggaaaccgaacacggcgagccagatcccgaagacgtgctgcgcgaaatcaacggctactatctggatggcccgaagaaggggcagctgctgcctggctttacagagatgaagcctgatggcacgacgtctggtggctgctggatctactccggcgtgttcaaggacaacatcaaccagtccgcgcgcaaagtttcaggcgcttcgcaaaatgaggttgcgctggaatggggctgggtatggccatcgaatcgccgcatgctgtacaaccgtgcgtcagctgcgccagacggcacgccatggtcggagcgcaagaagtacatttggtgggacgctgaggccggccgctggacgggcgacgacgtaccggacttcccagtcaacttggatccgtcataccgcgcgcctgtcgatgccacaggtcctgcagcccttgacggcaccgatgcgtttatcatgcaggcagatggtcgtggttggttgttcgtacccaaaggactttccgatggacccctgccaacccactatgaaccgcacgagtcgccggcacgcaatattttgtacagccagcagcagtcgccgacacgcttgaccatcaagcgtccggataacttgtcgaagcccatggctggtgagcccggctcagaggtctaccccgtggttttctccacgtaccgtttgacggagatgtacacctcgggtgcgatgagccgccgactgccttatttggcagagttgcagccagatttgttcgttgaggtcgatccggttctagcacaaaagcgcggcttggaaaacggtggctgggcaaccatcatttcgccgcgtggcgtgattgaggctcgcgtgctggtgaccgaacgcatggaatctatgaccatcaatggcaaggacttccaccagattggtctgcctttccactacggtcagtccagctcctcgccagttactggtgacggtgccaatgaccttctgggtctaactttggagccgaatgtgttcattcaaaactccaaggttggtgcatgtgaaattaaggccggccgacgcccacgcggcaaggcgcggttagagatgctcaaggaataccagcgccgtgccggattgacgttggacaccggtaacgagctcatcgatcccgatgcacagcagctcgaagctacctccacgatcgacttatttattccgaatggcgtagacaaagagacggtggagacatcgacaagcgagcctggcgccgcagatggttctgcgcatcatggctcagcgatgggggaagtcccaaattctgaaccaaaagatacggagggaggcgaaaagcaatga

SEQ ID NO: 57 - protein, 188 aa, Corynebacterium stationis
MSKLSPLNWPVVRQVKRGDLFGRDKSTQSAKSENLHGRTVEADKVVQSVCPYCAVGCSQRVYVKDDRVVHIEGDSDSPISRGRLCPKGAASEQLVNSATRLTKIKYRAPHATEWQDLDLETAMDMIADRFIASRRNQWQDFDEKGRVLNRTMGVAGLGGATLDNEENYIIKKLFTAAGAVQVENQARI

SEQ ID NO: 58 - DNA, 567 bp, Corynebacterium stationis
  source 1..567: mol_type = genomic DNA
atgtcgaagttaagtccgctgaattggccggttgtgcgccaggtgaagcgcggcgatctgtttggtcgagataaatcaacccagtctgccaaatcggagaacctgcacgggcgcactgtagaggccgacaaagtagttcaatcggtctgcccttactgcgctgtgggctgctcgcagcgggtatatgtcaaagatgaccgcgtcgttcatattgaaggtgactcggactcgcctatttcgcgcggacgtttgtgcccgaaaggcgctgcctctgagcagctggtgaactctgcgacgcgtttgaccaagattaaataccgcgcgcctcatgcaaccgagtggcaagacctagatctcgaaaccgcaatggatatgattgcggaccgttttattgcctcccgccgcaatcagtggcaggactttgatgaaaaaggccgtgttttaaaccgcaccatgggtgtggcaggacttggtggcgccaccttggataatgaggaaaactacattatcaagaagctgtttactgcagctggtgccgtacaagtcgaaaaccaagcacgcatatga